European Patent Specification EP 4 164 784 B1, published June 25, 2025. Title: SYSTEMS, APPARATUS AND KITS FOR ENZYMATIC POLYNUCLEOTIDE SYNTHESIS. Applicant: DNA Script. The sequence listing filed with the application follows.

SEQUENCE LISTING (71 sequences)

SEQ ID NO: 1 - protein, 510 aa, mouse
MDPLQAVHLGPRKKRPRQLGTPVASTPYDIRFRDLVLFILEKKMGTTRRAFLMELARRKGFRVENELSDSVTHIVAENNSGSDVLEWLQLQNIKASSELELLDISWLIECMGAGKPVEMMGRHQLVVNRNSSPSPVPGSQNVPAPAVKKISQYACQRRTTLNNYNQLFTDALDILAENDELRENEGSCLAFMRASSVLKSLPFPITSMKDTEGIPCLGDKVKSIIEGIIEDGESSEAKAVLNDERYKSFKLFTSVFGVGLKTAEKWFRMGFRTLSKIQSDKSLRFTQMQKAGFLYYEDLVSCVNRPEAEAVSMLVKEAVVTFLPDALVTMTGGFRRGKMTGHDVDFLITSPEATEDEEQQLLHKVTDFWKQQGLLLYCDILESTFEKFKQPSRKVDALDHFQKCFLILKLDHGRVHSEKSGQQEGKGWKAIRVDLVMCPYDRRAFALLGWTGSRQFERDLRRYATHERKMMLDNHALYDRTKRVFLEAESEEEIFAHLGLDYIEPWERNA

SEQ ID NO: 2 - protein, 381 aa, mouse
NSSPSPVPGSQNVPAPAVKKISQYACQRRTTLNNYNQLFTDALDILAENDELRENEGSCLAFMRASSVLKSLPFPITSMKDTEGIPCLGDKVKSIIEGIIEDGESSEAKAVLNDERYKSFKLFTSVFGVGLKTAEKWFRMGFRTLSKIQSDKSLRFTQMQKAGFLYYEDLVSCVNRPEAEAVSMLVKEAVVTFLPDALVTMTGGFRRGKMTGHDVDFLITSPEATEDEEQQLLHKVTDFWKQQGLLLYCDILESTFEKFKQPSRKVDALDHFQKCFLILKLDHGRVHSEKSGQQEGKGWKAIRVDLVMCPYDRRAFALLGWTGSRQFERDLRRYATHERKMMLDNHALYDRTKRVFLEAESEEEIFAHLGLDYIEPWERNA

SEQ ID NO: 3 - protein, 380 aa, bovine
DYSATPNPGFQKTPPLAVKKISQYACQRKTTLNNYNHIFTDAFEILAENSEFKENEVSYVTFMRAASVLKSLPFTIISMKDTEGIPCLGDKVKCIIEEIIEDGESSEVKAVLNDERYQSFKLFTSVFGVGLKTSEKWFRMGFRSLSKIMSDKTLKFTKMQKAGFLYYEDLVSCVTRAEAEAVGVLVKEAVWAFLPDAFVTMTGGFRRGKKIGHDVDFLITSPGSAEDEEQLLPKVINLWEKKGLLLYYDLVESTFEKFKLPSRQVDTLDHFQKCFLILKLHHQRVDSSKSNQQEGKTWKAIRVDLVMCPYENRAFALLGWTGSRQFERDIRRYATHERKMMLDNHALYDKTKRVFLKAESEEEIFAHLGLDYIEPWERNA

SEQ ID NO: 4 - protein, 380 aa, human
DYSDSTNPGPPKTPPIAVQKISQYACQRRTTLNNCNQIFTDAFDILAENCEFRENEDSCVTFMRAASVLKSLPFTIISMKDTEGIPCLGSKVKGIIEEIIEDGESSEVKAVLNDERYQSFKLFTSVFGVGLKTSEKWFRMGFRTLSKVRSDKSLKFTRMQKAGFLYYEDLVSCVTRAEAEAVSVLVKEAVWAFLPDAFVTMTGGFRRGKKMGHDVDFLITSPGSTEDEEQLLQKVMNLWEKKGLLLYYDLVESTFEKLRLPSRKVDALDHFQKCFLIFKLPRQRVDSDQSSWQEGKTWKAIRVDLVLCPYERRAFALLGWTGSRQFERDLRRYATHERKMILDNHALYDKTKRIFLKAESEEEIFAHLGLDYIEPWERNA

SEQ ID NO: 5 - protein, 376 aa, chicken
QYPTLKTPESEVSSFTASKVSQYSCQRKTTLNNCNKKFTDAFEIMAENYEFKENEIFCLEFLRAASVLKSLPFPVTRMKDIQGLPCMGDRVRDVIEEIIEEGESSRAKDVLNDERYKSFKEFTSVFGVGVKTSEKWFRMGLRTVEEVKADKTLKLSKMQRAGFLYYEDLVSCVSKAEADAVSSIVKNTVCTFLPDALVTITGGFRRGKKIGHDIDFLITSPGQREDDELLHKGLLLYCDIIESTFVKEQIPSRHVDAMDHFQKCFAILKLYQPRVDNSSYNMSKKCDMAEVKDWKAIRVDLVITPFEQYAYALLGWTGSRQFGRDLRRYATHERKMMLDNHALYDKRKRVFLKAGSEEEIFAHLGLDYVEPWERNA

SEQ ID NO: 6 - protein, 387 aa, possum
SANPDPTAGTLNILPPTTKTISQYACQRRTTINNHNQRFTDAFEILAKNYEFKENDDTCLTFMRAISVLKCLPFEVVSLKDTEGLPWIGDEVKGIMEEIIEDGESLEVQAVLNDERYQSFKLFTSVFGVGLKTADKWYRMGFRTLNKIRSDKTLKLTKMQKAGLCYYEDLIDCVSKAEADAVSLLVQDAVWTFLPDALVTITGGFRRGKEFGHDVDFLITSPGAEKEQEDQLLQKVTNLWKKQGLLLYCDLIESTFEDLKLPSRKIDALDHFQKCFLILKLYHHKEDKRKWEMPTGSNESEAKSWKAIRVDLVVCPYDRYAFALLGWSGSRQFERDLRRYATHEKKMMLDNHALYDKTKKIFLKAKSEEEIFAHLGLEYIQPSERNA

SEQ ID NO: 7 - protein, 381 aa, shrew
DCPASHDSSPQKTESAAVQKISQYACQRRTTLNNHNHIFTDAFEILAENCEFRENEGSYVTYMRAASVLKSLPFSIISMKDTEGIPCLADKVKCVIEEIIEDGESSEVKAVLNDERYKSFKLFTSVFGVGLKTAEKWFRLGFRTLSGIMNDKTLKLTHMQKAGFLYYEDLVSCVTRAEAEAVGVLVKEAVWAFLPDAIVTMTGGFRRGKKVGHDVDFLITSPEATEEQEQQLLHKVITFWEKEGLLLYCDLYESTFEKLKMPSRKVDALDHFQKCFLILKLHRECVDDGTSSQLQGKTWKAIRVDLVVCPYECRAFALLGWTGSPQFERDLRRYATHERKMMLDNHALYDKTKRKFLSADSEEDIFAHLGLDYIEPWERNA

SEQ ID NO: 8 - protein, 381 aa, dog
DYTASPNPELQKTLPVAVKKISQYACQRRTTLNNYNNVFTDAFEVLAENYEFRENEVFSLTFMRAASVLKSLPFTIISMKDTEGIPCLGDQVKCIIEEIIEDGESSEVKAVLNDERYQSFKLFTSVFGVGLKTSEKWFRMGFRTLSKIKSDKSLKFTPMQKAGFLYYEDLVSCVTRAEAEAVGVLVKEAVGAFLPDAFVTMTGGFRRGKKMGHDVDFLITSPGSTDEDEEQLLPKVINLWERKGLLLYCDLVESTFEKLKLPSRKVDALDHFQKCFLILKLHHQRVDGGKCSQQEGKTWKAIRVDLVMCPYERRAFALLGWTGSRQFERDLRRYASHERKMILDNHALYDKTKKIFLKAESEEEIFAHLGLDYIEPWERNA

SEQ ID NO: 9 - protein, 382 aa, mole
GDCPASHDSSPQKTESAAVQKISQYACQRRTTLNNHNHIFTDAFEILAENCEFRENEGSYVTYMRAASVLKSLPFSIISMKDTEGIPCLADKVKCVIEEIIEDGESSEVKAVLNDERYKSFKLFTSVFGVGLKTAEKWFRLGFRTLSGIMNDKTLKLTHMQKAGFLYYEDLVSCVTRAEAEAVGVLVKEAVWAFLPDAIVTMTGGFRRGKKVGHDVDFLITSPEATEEQEQQLLHKVITFWEKEGLLLYCDLYESTFEKLKMPSRKVDALDHFQKCFLILKLHRECVDDGTSSQLQGKTWKAIRVDLVVCPYECRAFALLGWTGSPQFERDLRRYATHERKMMLDNHALYDKTKRKFLSADSEEDIFAHLGLDYIEPWERNA

SEQ ID NO: 10 - protein, 379 aa, pika
EYSANPSPGPQATPAVYKISQYACQRRTTLNNHNHIFTDAFEILAENYEFKENEGCYVTYMRAASVLKSLPFTIVSMKDTEGIPCLEDKVKSIMEEIIEEGESSEVKAVLSDERYQCFKLFTSVFGVGLKTSEKWFRMGFRSLSNIRLDKSLKFTQMQKAGFRYYEDIVSCVTRAEAEAVDVLVNEAVRAFLPDAFITMTGGFRRGKKIGHDVDFLITSPELTEEDEQQLLHKVMNLWEKKGLLLYHDLVESTFEKLKQPSRKVDALDHFQKCFLIFKLYHERVGGDRCRQPEGKDWKAIRVDLVMCPYECHAFALLGWTGSRQFERDLRRYASHERKMILDNHALYDKTKRVFLQAENEEEIFAHLGLDYIEPWERNA

SEQ ID NO: 11 - protein, 384 aa, hedgehog
DASFGSNPGSQNTPPLAIKKISQYACQRRTSLNNCNHIFTDALDILAENHEFRENEVSCVAFMRAASVLKSLPFTIISMKDTKGIPCLGDKAKCVIEEIIEDGESSEVKAILNDERYQSFKLFTSVFGVGLKTSEKWFRMGFRTLNKIMSDKTLKLTRMQKAGFLYYEDLVSCVAKAEADAVSVLVQEAVWAFLPDAMVTMTGGFRRGKKLGHDVDFLITSPGATEEEEQQLLPKVINFWERKGLLLYHDLVESTFEKLKLPSRKVDALDHFQKCFLILKLHLQHVNGVGNSKTGQQEGKNWKAIRVDLVMCPYERRAFALLGWTGSRQFERDLRRFATHERKMMLDNHALYDKTKRIFLKAESEEEIFAHLGLDYIDPWERNA

SEQ ID NO: 12 - protein, 381 aa, tree shrew
DHSTSPSPGPQKTPALAVQKISQYACQRRTTLNNCNRVFTDAFETLAENYEFRENEDSSVIFLRAASVLRSLPFTITSMRDTEGLPCLGDKVKCVIEEIIEDGESSEVNAVLNDERYKSFKLFTSVFGVGLKTSEKWFRMGFRTLSRVRSDKSLHLTRMQQAGFLYYEDLASCVTRAEAEAVGVLVKEAVGAFLPDALVTITGGFRRGKKTGHDVDFLITSPGSTEEKEEELLQKVLNLWEKKGLLLYYDLVESTFEKLKTPSRKVDALDHFPKCFLILKLHHQRVDGDKPSQQEGKSWKAIRVDLVMCPYERHAFALLGWTGSRQFERDLRRYATHERKMMLDNHALYDKTKRVFLKAESEEDIFAHLGLDYIEPWERNA

SEQ ID NO: 13 - protein, 394 aa, platypus
LTNSAPINCMTETPSLATKQVSQYACERRTTLNNCNQKFTDAFEILAKDFEFRENEGICLAFMRAISVLKCLPFTIVRMKDIEGVPWLGDQVKSIIEEIIEDGESSSVKAVLNDERYRSFQLFNSVFEVGLTDNGENGIARGFQTLNEVITDENISLTKTTLSTSLWNYLPGFLYYEDLVSCVAKEEADAVYLIVKEAVRAFLPEALVTLTGGFRRGKKIGHDVDFLISDPESGQDEQLLPNIIKLWEKQELLLYYDLVESTFEKTKIPSRKVDAMDHFQKCFLILKLHHQKVDSGRYKPPPESKNHEAKNWKAIRVDLVMCPFEQYAYALLGWTGSRQFERDLRRYATHEKKMMLDNHALYDKTKKIFLKAESEEDIFTHLGLDYIEPWERNA

SEQ ID NO: 14 - protein, 384 aa, jerboa
SSELELLDVSWLIECMGAGKPVEMTGRHQLVKQTFCLPGFILQDAFDILAENCEFRENEASCVEFMRAASVLKSLPFPIISVKDTEGIPWLGGKVKCVIEEIIEDGESSEVKALLNDERYKSFKLFTSVFGVGLKTAERWFRMGFRTLSTVKLDKSLTFTRMQKAGFLHYEDLVSCVTRAEAEAVSVLVQQAVVAFLPDALVSMTGGFRRGKKIGHDVDFLITSPEATEEEEQQLLHKVTNFWEQKGLLLYCDHVESTFEKCKLPSRKVDALDHFQKCFLILKLYRERVDSVKSSQQEGKGWKAIRVDLVMCPYECRAFALLGWTGSRQFERDLRRYATHERKMRLDNHALYDKTKRVFLKAESEEEIFAHLGLEYIEPLERNA

SEQ ID NO: 15 - protein, 364 aa, puma
VVKKIPLYACQRRTTLNNFNHIFTDAFEVLAENYEFKENEISSATFMRAASVLKLPFTIISMKDTEGIPCLGDKVKCVIEEIIEDGESSEVKAVLNDERYQSFKLFTSVFGVGLKTSEKWFRMGFRTLSKIKSDKTLKFTQMQKAGFLYYEDLVSCVTRAEAEAVGVLVKEAVWAFLPDAFVTMTGGFRRGKKIGHDVDFLITIPGSTDEEEEQLLPKVINLWQRKELLLYYDLVESTFEKLKLPSRKVDALDHFQKCFLILKLHHQRVDSGKCSQQEGKTWKAIRVDLVMCPYERRAFALLGWTGSRQFERDLRRYATHERKMILDNHALYDKTKKIFLKAESEEEIFAHLGLDYIEPWERNA

SEQ ID NO: 16 - protein, 362 aa, mouse
KISQYACQRRTTLNNYNQLFTDALDILAENDELRENEGSCLAFMRASSVLKSLPFPITSMKDTEGIPCLGDKVKSIIEGIIEDGESSEAKAVLNDERYKSFKLFTSVFGVGLKTAEKWFRMGFRTLSKIQSDKSLRFTQMQKAGFLYYEDLVSCVNRPEAEAVSMLVKEAVVTFLPDALVTMTGGFRRGKMTGHDVDFLITSPEATEDEEQQLLHKVTDFWKQQGLLLYCDILESTFEKFKQPSRKVDALDHFQKCFLILKLDHGRVHSEKSGQQEGKGWKAIRVDLVMCPYDRRAFALLGWTGSRQFERDLRRYATHERKMMLDNHALYDRTKRVFLEAESEEEIFAHLGLDYIEPWERNA

SEQ ID NO: 17 - protein, 361 aa, Bovine
KISQYACQRKTTLNNYNHIFTDAFEILAENSEFKENEVSYVTFMRAASVLKSLPFTIISMKDTEGIPCLGDKVKCIIEEIIEDGESSEVKAVLNDERYQSFKLFTSVFGVGLKTSEKWFRMGFRSLSKIMSDKTLKFTKMQKAGFLYYEDLVSCVTRAEAEAVGVLVKEAVWAFLPDAFVTMTGGFRRGKKIGHDVDFLITSPGSAEDEEQLLPKVINLWEKKGLLLYYDLVESTFEKFKLPSRQVDTLDHFQKCFLILKLHHQRVDSSKSNQQEGKTWKAIRVDLVMCPYENRAFALLGWTGSRQFERDIRRYATHERKMMLDNHALYDKTKRVFLKAESEEEIFAHLGLDYIEPWERNA

SEQ ID NO: 18 - protein, 361 aa, Human
KISQYACQRRTTLNNCNQIFTDAFDILAENCEFRENEDSCVTFMRAASVLKSLPFTIISMKDTEGIPCLGSKVKGIIEEIIEDGESSEVKAVLNDERYQSFKLFTSVFGVGLKTSEKWFRMGFRTLSKVRSDKSLKFTRMQKAGFLYYEDLVSCVTRAEAEAVSVLVKEAVWAFLPDAFVTMTGGFRRGKKMGHDVDFLITSPGSTEDEEQLLQKVMNLWEKKGLLLYYDLVESTFEKLRLPSRKVDALDHFQKCFLIFKLPRQRVDSDQSSWQEGKTWKAIRVDLVLCPYERRAFALLGWTGSRQFERDLRRYATHERKMILDNHALYDKTKRIFLKAESEEEIFAHLGLDYIEPWERNA

SEQ ID NO: 19 - protein, 358 aa, Chicken
KVSQYSCQRKTTLNNCNKKFTDAFEIMAENYEFKENEIFCLEFLRAASVLKSLPFPVTRMKDIQGLPCMGDRVRDVIEEIIEEGESSRAKDVLNDERYKSFKEFTSVFGVGVKTSEKWFRMGLRTVEEVKADKTLKLSKMQRAGFLYYEDLVSCVSKAEADAVSSIVKNTVCTFLPDALVTITGGFRRGKKIGHDIDFLITSPGQREDDELLHKGLLLYCDIIESTFVKEQIPSRHVDAMDHFQKCFAILKLYQPRVDNSSYNMSKKCDMAEVKDWKAIRVDLVITPFEQYAYALLGWTGSRQFGRDLRRYATHERKMMLDNHALYDKRKRVFLKAGSEEEIFAHLGLDYVEPWERNA

SEQ ID NO: 20 - protein, 368 aa, Possum
TISQYACQRRTTINNHNQRFTDAFEILAKNYEFKENDDTCLTFMRAISVLKCLPFEVVSLKDTEGLPWIGDEVKGIMEEIIEDGESLEVQAVLNDERYQSFKLFTSVFGVGLKTADKWYRMGFRTLNKIRSDKTLKLTKMQKAGLCYYEDLIDCVSKAEADAVSLLVQDAVWTFLPDALVTITGGFRRGKEFGHDVDFLITSPGAEKEQEDQLLQKVTNLWKKQGLLLYCDLIESTFEDLKLPSRKIDALDHFQKCFLILKLYHHKEDKRKWEMPTGSNESEAKSWKAIRVDLVVCPYDRYAFALLGWSGSRQFERDLRRYATHEKKMMLDNHALYDKTKKIFLKAKSEEEIFAHLGLEYIQPSERNA

SEQ ID NO: 21 - protein, 362 aa, shrew
KISQYACQRRTTLNNHNHIFTDAFEILAENCEFRENEGSYVTYMRAASVLKSLPFSIISMKDTEGIPCLADKVKCVIEEIIEDGESSEVKAVLNDERYKSFKLFTSVFGVGLKTAEKWFRLGFRTLSGIMNDKTLKLTHMQKAGFLYYEDLVSCVTRAEAEAVGVLVKEAVWAFLPDAIVTMTGGFRRGKKVGHDVDFLITSPEATEEQEQQLLHKVITFWEKEGLLLYCDLYESTFEKLKMPSRKVDALDHFQKCFLILKLHRECVDDGTSSQLQGKTWKAIRVDLVVCPYECRAFALLGWTGSPQFERDLRRYATHERKMMLDNHALYDKTKRKFLSADSEEDIFAHLGLDYIEPWERNA

SEQ ID NO: 22 - protein, 362 aa, dog
KISQYACQRRTTLNNYNNVFTDAFEVLAENYEFRENEVFSLTFMRAASVLKSLPFTIISMKDTEGIPCLGDQVKCIIEEIIEDGESSEVKAVLNDERYQSFKLFTSVFGVGLKTSEKWFRMGFRTLSKIKSDKSLKFTPMQKAGFLYYEDLVSCVTRAEAEAVGVLVKEAVGAFLPDAFVTMTGGFRRGKKMGHDVDFLITSPGSTDEDEEQLLPKVINLWERKGLLLYCDLVESTFEKLKLPSRKVDALDHFQKCFLILKLHHQRVDGGKCSQQEGKTWKAIRVDLVMCPYERRAFALLGWTGSRQFERDLRRYASHERKMILDNHALYDKTKKIFLKAESEEEIFAHLGLDYIEPWERNA

SEQ ID NO: 23 - protein, 362 aa, MOLE; identical to SEQ ID NO: 21

SEQ ID NO: 24 - protein, 362 aa, Pika
KISQYACQRRTTLNNHNHIFTDAFEILAENYEFKENEGCYVTYMRAASVLKSLPFTIVSMKDTEGIPCLEDKVKSIMEEIIEEGESSEVKAVLSDERYQCFKLFTSVFGVGLKTSEKWFRMGFRSLSNIRLDKSLKFTQMQKAGFRYYEDIVSCVTRAEAEAVDVLVNEAVRAFLPDAFITMTGGFRRGKKIGHDVDFLITSPELTEEDEQQLLHKVMNLWEKKGLLLYHDLVESTFEKLKQPSRKVDALDHFQKCFLIFKLYHERVGGDRCRQPEGKDWKAIRVDLVMCPYECHAFALLGWTGSRQFERDLRRYASHERKMILDNHALYDKTKRVFLQAENEEEIFAHLGLDYIEPWERNA

SEQ ID NO: 25 - protein, 365 aa, TRUNC HEDGEHOG
KISQYACQRRTSLNNCNHIFTDALDILAENHEFRENEVSCVAFMRAASVLKSLPFTIISMKDTKGIPCLGDKAKCVIEEIIEDGESSEVKAILNDERYQSFKLFTSVFGVGLKTSEKWFRMGFRTLNKIMSDKTLKLTRMQKAGFLYYEDLVSCVAKAEADAVSVLVQEAVWAFLPDAMVTMTGGFRRGKKLGHDVDFLITSPGATEEEEQQLLPKVINFWERKGLLLYHDLVESTFEKLKLPSRKVDALDHFQKCFLILKLHLQHVNGVGNSKTGQQEGKNWKAIRVDLVMCPYERRAFALLGWTGSRQFERDLRRFATHERKMMLDNHALYDKTKRIFLKAESEEEIFAHLGLDYIDPWERNA

SEQ ID NO: 26 - protein, 362 aa, tree shrew
KISQYACQRRTTLNNCNRVFTDAFETLAENYEFRENEDSSVIFLRAASVLRSLPFTITSMRDTEGLPCLGDKVKCVIEEIIEDGESSEVNAVLNDERYKSFKLFTSVFGVGLKTSEKWFRMGFRTLSRVRSDKSLHLTRMQQAGFLYYEDLASCVTRAEAEAVGVLVKEAVGAFLPDALVTITGGFRRGKKTGHDVDFLITSPGSTEEKEEELLQKVLNLWEKKGLLLYYDLVESTFEKLKTPSRKVDALDHFPKCFLILKLHHQRVDGDKPSQQEGKSWKAIRVDLVMCPYERHAFALLGWTGSRQFERDLRRYATHERKMMLDNHALYDKTKRVFLKAESEEDIFAHLGLDYIEPWERNA

SEQ ID NO: 27 - protein, 375 aa, TRUNCATED PLATYPUS
QVSQYACERRTTLNNCNQKFTDAFEILAKDFEFRENEGICLAFMRAISVLKCLPFTIVRMKDIEGVPWLGDQVKSIIEEIIEDGESSSVKAVLNDERYRSFQLFNSVFEVGLTDNGENGIARGFQTLNEVITDENISLTKTTLSTSLWNYLPGFLYYEDLVSCVAKEEADAVYLIVKEAVRAFLPEALVTLTGGFRRGKKIGHDVDFLISDPESGQDEQLLPNIIKLWEKQELLLYYDLVESTFEKTKIPSRKVDAMDHFQKCFLILKLHHQKVDSGRYKPPPESKNHEAKNWKAIRVDLVMCPFEQYAYALLGWTGSRQFERDLRRYATHEKKMMLDNHALYDKTKKIFLKAESEEDIFTHLGLDYIEPWERNA

SEQ ID NO: 28 - protein, 365 aa, Serinus canaria
KVSQYSCQRKTTLNNYNKKFTDAFEVMAENYEFKENEIFCLEFLRAASLLKSLPFSVTRMKDIQGLPCMGDQVRDVIEIIEEGESSRVKEVLNDERYKAFKQFTSVFGVGVKTSEKWYRMGLRTVGEVKADKTLKLSKMQKAGFLYYEDLVSCVSKAEADAVSLIVKNTVCTFLPDALVTITGGFRRGKNIGHDIDFLITNPGPREDDELLHKVIDLWKKQGLLLYCDIIESTFVKEQLPSRKIDAMDHFQKCFAILKLYQPRVDNSTCNTSKKLEMAEVKDWKAIRVDLVITPFEQYSYALLGWTGSRQFGRDLRRYAAHERRMILDNHGLYDRTKRIFLKAGSEEEIFAHLGLDYVEPWERNA

SEQ ID NO: 29 - protein, 366 aa, Neopelma chrysocephalum
KVSQYSCQRKTTLNNYNKKFTDAFEIMAENYEFKENEIFCLEFLRAASLLKYLPFPVTRMKDIQGLPCIGDQVRDVIEGIIEEGESSRVKEVLNDERYKAFKQFTSVFGVGVKTSEKWYRMGLRTVEELKADKTLKLSKMQKAGFLYYEDLVSCVSKAEADAVTLIVKNTVSTFLPDALVTITGGFRRGKKMGHDIDFLITNPGPREDDELLHKVVDLWKKQGLLLYCDIIESTFVEEQLPSRKVDAMDNFQKCFTILKLYQPGVDNSSYNMSKKSDMAEVKDWKAIRVDLVITPFEQYAYALLGWTGSREFGRDLRRYASHERKMILDNHGLYDRRKRIFLKAGSEEEIFAHLGLDYVEPWERNA

SEQ ID NO: 30 - protein, 366 aa, Alligator sinensis
KVSQYACQRRTTLNNYNKKFTDAFEILAENCEFRENRLGCLEFLRAASVLKFLPFPIVKMKNIEGLPCMGDKVKCVIEEILEEGESCQAKEILNDERYKSFKLFTSVFGVGLKTTEKWYRMGFRTLEEVKAEKTLKLSRMQIAGFLHYEDIISYVSKAEADAVSLLIKDTVCMFLPDALVTITGGFRRGKKTGHDVDFLITNPGPEEEKELLHKVVDLWEKQGLLLYYDVIESTFEKEKRPSRKVDALDHFQKCFAILKLHQQRRGNSNSNISKESDKAEVKDWKAIRVDLVISPFEQYAYALLGWTGSRQFERDLRRYASRERKMMLDNHALYDKTKRTFLKAESEEEIFAHLGLDYIEPWERNA

SEQ ID NO: 31 - protein, 366 aa, Alligator sinensis
KISEYACQRRTTLNNYNKKFTDAFEILAENYEFNENKGFCLAFRRAASVLKFLPFTIVRMNDIQGLPWMGDQVKRVIEEILEEGESSKVKEVLNDEKYKAFKLFTSVFGVGRKTSEKWYRMGLRTLEEVKADKTLKLTKMQKAGFLYYEDLISRVSKAEADAVSLIVKDTVWKFLPDALVTLTGGFRLGKKMGHDVDFLITTPGPEEEEELLHKVIDLWKKQGLLLYYDIIESTFEKTKLPSRTVDALDHFQKCFAILKLHKQRVDNGNSNQSKEFDKEETKDWKAIRVDLVITPFEQYAYALLGWTGSAFFNRDLRRYATHEKKMMLDNHALYDKTKRIFLKAASEEEIFAHLGLDYLEPWERNA

SEQ ID NO: 32 - protein, 363 aa, Xenopus laevis
KVSQYACQRCTTLQDTNRIFTDAFDILAEHFEFCENKGRTVAFLRASSLIKSLPFPITAMKELEGLPWLGDQMKGIIEEILEEGKSYKVLEVMNEERYKSFKQFTSVFGVGLKTSDKWFRMGFRTLEEIKNEKELKLTKMQKCGLLYYEDITSYVSRAEAETTEQLIKSIVWKFVPDAIVTLTGGFRRGKKKGHDVDILITCARKGKEKNILHNTMSVLKNRGLLLFYNIIESTFDETKLPSRHVDALDHFQKCFTILKLPKRQMDIGNIIDPHECERKNWKAVRLDLVITPYEQYPYALLGWTGSRQFERDLRRYATHEKRMMLDNHGLYDKTKNNFLKANNEEDIFKQLGLDYLEPWERNA

SEQ ID NO: 33 - protein, 363 aa, Xenopus
KVSEYACQRRTTLQDTNRIFTDAFDILAENYEFNENKGPCVAFRRASSVLKSLPFPIVAMKDLEGLPWLGDQMKRIIEEILEEGKSSKVVEVMNDERYKAFKLFTSVFGVGRKTSEKWFRMGFRTLEEIKSDKELKLTKMQKAGLLYYEDITSAVSKAEAEAVEQLIKSIVWKFVPDAIVTLTGGFRLGKKMGHDVDILITTPRKGEKEEILHKTINVLKKRGLLLFYNIIESTFDETKLPSRHVDALDHFQKCFTILKLQKQQLDNGNSNEPFETEKKNWKAIRVDLVITPYEQYAYALLGWTGSPQFNRDLRRYATHEKRMMLDNHALYDKTKNIFLKANSEEDIFTHLGLDYLEPWERNA

SEQ ID NO: 34 - protein, 367 aa, Notechis
SISEYACQRRTTLNNYNKKFTDAFEILAENYEFNENKGFCLAFRRAASVLKFLPFTIVRVNDIEGLPWMGEQVKRIIEDILEEGESSKVKAVLNNENYRAFKLFTSVFGVGRKTSEKWYRMGLRTLEEVKADKNLKLTRMQKAGFLHYEDLISRVSKAEADAASLIVKDTVWKFLPNALVTLTGGFRLGKKMGHDVDFLITVPGSRQEEEELLHTVIDLWKKQGLLLYYDLIESTFEKTKLPSRTVDALDHFQKCFAILKLHKERVDKGNSIQSKAFAEEETKDWKAIRVDLVVTPFEQYAFALLGWTGSPFFNRDLRRYATHEKKMMLDNHALYDKTKKIFLKAASEEEIFAHLGLDYLEPWERNA

SEQ ID NO: 35 - protein, 363 aa, Salmo trutta
NVSQYACLRRTTTENHNKIFTDVLEELAENSEFNESKGPCLAFRRAASVLKSLPSAVHCLGAIQGLPCLGEHTKAVMEEILIFGRSFKVEEVQSDERYQALKLFTSVFGVGPKTAEKWYRRGLRSLKEILAEPNIQLNRMQRAGFLYYRDISKAVSKAEAKALSSIIEETAHWIAPDSILALTGGFRRGKEYGHDVDFLLTMPEMGKEEGLLLRVIDRLRDQGILLYCEHQDSTFDMSKLPSHRFEAMDHFEKCFLILRLEEGQVEGDGGLQKDPGESRGWRAVRVDLVAPPVDRYAFVLLGWTGSRQFERDLRRFASKERGMCLDNHALYDKTKKLFLPATSEEDIFAHLGLEYVEPWQRNA

SEQ ID NO: 36 - protein, 363 aa, Salmo trutta
TVSEYACQRRTTMENHNKIFTDAFEVLAENSEFNESKESRDAFRRAASVLKSLPSAVRSLGDTEGLPCLGEHTKRVIEEILEYGRSSKVEDILSDERYQTMKLFTSVFGVGPKTAEKWYRRGLRSLEEVRAEPSIHLNRMQRAGFLYYRDISKRVSKAEAKALGNIIEETVHAIAPDAIVTLTGGFRLGKEFGHDVDFILTTPEMGKEEGLLPRVIDRLRNQGILLYCDYQESTFDMSKLPSRTFEAMDHFQKCFLIIKLKEGLVEGEGGLQSDPGDRRGWRAVRVDLVAPPVDRYAFALLGWTGSPQFNRDLRRFARLERRMLLDNHALYDKTKKIFLPAKTEEDIFAHLGLEYIEPWQRNA

SEQ ID NO: 37 - protein, 360 aa, Electrophorus electricus
TVSQYACQRRTTLDNHNKVFTDALEVLIENYEFSDNKGACVGFRRAASVLKSLPKPLRCLKDMEGLPCLGDDTKAIIEEIYECGSSSRVENILSDEKYQTLKLFTSVFGVGPKTGEKWYRRGLRALEQVHSEPSIQLNKMQAAGFLYYEDISKPVSRAEAKAVGCIIEEVASCFSSSVTITLTGGFRRGKEFGHDVDFLLSIPEPGKEDGLLPAVIDRLRKQGILLYSDLQESTLQQWKRPSRCFDSMDHFQKCFLIVKLWTRLVEGHREDPSSQRDWKAVRVDLVVPPVDCYAFALLGWSGSTQFERDLRRFARLERRMLLDNHALYDKTTNTFLQAKTEEDIFAHLGLDYIEPWQRNA

SEQ ID NO: 38 - protein, 360 aa, Electrophorus electricus
TVSEYACQRRTTLDNHNKIFTDALEVLAENYEFSDSKESRDAFRRAASVLKSLPTPLRSLQDTEGLPCLGEETKRVIEEIFEEGSSSRVEDILSDERYQTLKLFTSVFGVGPKTAEKWYRRGLRSLEQVRSDPSIHLNRMQTAGFLYYEDISKPVSKAEAKALGNIIEETASAFSPSVTITLTGGFRLGKEFGHDVDFLLTVPEPGKEDGLLPAVIDRLRSQGILLYSDFQESTFDLSKLPSRRFEAMDHFQKCFLIVKLKAGLVEGEGADPGDRRDWRAVRVDLVAPPVDRYAFALLGWSGSAFFNRDLRRFARLERGMLLDNHALYDKTTNTFLQAKTEEDIFAHLGLDYIEPWQRNA

SEQ ID NO: 39 - protein, 361 aa, Anabas testudineus
TVSQYACQRRTTTENNNKILTDAFEVLAESYELNQLEGPCLAFRRAASVLKSLPWAVQCLGATQGLPCLGEHTKALIEEILQYGHSFEVEKILSDERYQTLKLFTSVFGVGPKTAEKWYRRGLRSFSDILAEPSIQLNRMQQSGFLHYGDISRAVSKAEARALGNIIDEAVHAITPDGILALTGGFRRGKEFGHDVDFIVTTPEQGKEETLLPNIIDRLKEQGILLYSDYQTSTFDISKLPSHKFEAMDHFAKCFLILRLEGSLVDRGLNSTEGDSRGWRAVRVDLVSPPMERYAYALLGWTGSRQFERDLRRFARLEQHMLLDNHALYDKTKKEFLAATTERDIFAHLGLEYIEPWQRNA

SEQ ID NO: 40 - protein, 361 aa, Anabas testudineus
TVSEYACQRRTTTENNNKIFTDAFEVLAESYEFNEMEESRDAFRRAASVLKSLPWAVQSLGATQDLPCLGEHTKRVMEEILQYGRSFEVEKILSDERYQTLKLFTSVFGVGPKTAEKWYRRGLRSFEDIRAEPSIHLNRMQQSGFLHYGDISRAVSKAEARALGNIIDEAVHAITPDAILALTGGFRLGKEFGHDVDFIVTTPELGKEESLLPNIIDRLKKQGILLYSDYQASTFDMSKLPSHRFEAMDHFAKCFLILRLEGSQVEGGLNSAEGDSRGWRAVRVDLVSPPMDRYAFALLGWTGSAFFNRDLRRFARMERRMLLDNHALYDKTKKEFLAATTEKDIFAHLGLEYIEPWQRNA

SEQ ID NO: 41 - protein, 361 aa, Poecilia reticulate
KVSQYACQRRTTVENNNRIFTDAFEVLAENYEFNEIEGRCLAFRRAASVLKSLPWAVRSVGATLDLPCLGEHTTAVMKEILQYGRSFEVEKILSDERCQTLKLFTSVFGVGPKTAEKWYRRGLRSFSDVLAQPGIHLNRMQQSGFLHYGDISRAVSKAEARAVGNIIDEAVHVITPNAILALTGGFRRGKDFGHDVDFIVTTTELGKEKNLLISVIESLKKQGLLLFSDYQASTFDISKLPSHRFEAMDHFAKCFLILRLEGSRVEGGLQRAQADGRGWRAVRVDLVSPPADRFAFTMLGWTGSRMFERDLRRFARLERQMLLDNHALYDKTKKEFLTAATEKDIFDHLGLEYIEPWQRNA

SEQ ID NO: 42 - protein, 366 aa, artificial sequence; identical to SEQ ID NO: 31
  F57 trunc new (Poecilia reticulate) guppy  [56.66 percent identity to wt calc by NCBI BLASTP]

SEQ ID NO: 43 - protein, 362 aa, Rattus norvegicus
KISQYACQRRTTLNNHNQLFTDAFDILAENYEFRENEVSCLPFMRAASVLKSLSFPIVSMKDIEGIPCLGDKVKCVIEGIIEDGESSEVKAVLNDERYKSFKLFTSVFGVGLKTAEKWFRMGFRTLSKIKSDKSLRFTHMQKAGFLYYEDLVSCVNRAEAEAVSMLVKEAVVAFLPDALVTMTGGFRRGKMTGHDVDFLITSPEATEEEEQQLLHKVTNFWRQQGLLLYCDIIESTFEKFKLPSRKVDALDHFQKCFLILKLHRGLVRSEESGQQEGKDWKAIRVDLVMCPYERRAFALLGWTGSRQFERDLRRYATHERKMMLDNHALYDKTKRVFLEAESEEEIFAHLGLDYIEPWERNA

SEQ ID NO: 44 - protein, 366 aa, Rattus norvegicus
SVVEKISEYACQRRTTLNNHNEVFTRAFDILAENYEFRENEESRDAFRRASSVLKSLPFPIISMKDTEGIPCLGDKVKRVIEEIIEDGESSEVKAVLNDERYKAFKLFTSVFGVGRKTAEKWFRMGFRTLEKIKSDKSLRFTQMQKAGFLYYEDLAERVNRAEAEAIEMLVKEAVVAFLPDALVTMTGGFRLGKMTGHDVDFLITSPEATEEEEQQLLHKVTDFWRQQGLLLYCDIIESTFEKFKLPSRTVDALDHFQKCFLILKLHHGRVVSEKSGQQEGKGWKAIRVDLVMCPYERRAFALLGWTGSPFFNRDLRRYATHERKMMLDNHALYDKTKRVFLEAESEEEIFAHLGLDYIEPWERNA

SEQ ID NO: 45 - protein, 362 aa, Piliocolobus tephrosceles
KISQYACQRRTTLNNCNQIFTDAFDILAENCEFRENEDSCVTFMRAASVLKSLPFTIISMKDTEGIPCLGSKVKCIIEEIIEDGESSEVKAVLNDERYQSFKLFTSVFGVGLKTSEKWFRMGFRTLSKVRSDESLKFTRMQRAGFLYYEDLVSCVTRAEAEAVSALVKEAVWAFLPDAFVTMTGGFRRGKKMGHDVDFLITSPGSTEDEEQQLLQKVMNLWEKKGLLLYYDLVESTFEKLRLPSRKVDALDHFQKCFLIFKLPLQRVDSDQSSWQGGKTWKAIRVDLVMCPYERRAFALLGWTGSRQFERDLRRYATHERKMILDNHALYDKTKRIFLKAESEEEIFAHLGLDYIEPWERNA

SEQ ID NO: 46 - protein, 362 aa, Sus scrofa
KISQYACQRRTTLNNCNHIFTDAFEVLAENYEFRENETFCLAFMRAASVLKSLPFTIISMKDTEGIPCLGDKVKCVIEEIIEDGESSEVKAVLNDERYQSFKLFTSVFGVGLKTSERWFRMGFRSLSKIRSDKTLKFTRMQKAGFLYYEDLVSCVTRAEAEAVGVLVKEAVQAFLPDAFVTMTGGFRRGKKMGHDVDFLITSPGSTDDEEQQLLPKVVNLWEREGLLLYCDLVESTLEKSKLPSRNVDALDHFQKCFLILKLHHQRVDSGMSSQQEGKTWKAIRVDLVMCPYELRAFALLGWTGSRQFERDLRRYATHERKMILDNHALYDKTKRIFLKAESEEEIFAHLGLDYLEPWERNA

SEQ ID NO: 47 - protein, 362 aa, artificial sequence
  N27 trunc new  [88.13 percent identity to wt calc by NCBI BLASTP] pig
KISEYACQRRTTLNNYNEIFTRAFEILAENYEFRENEESYVTFRRAASVLKSLPFTIISMKDTEGIPCLGDKVKRVIEEIIEDGESSEVKAVLNDERYKAFKLFTSVFGVGRKTSEKWFRMGFRTLEKIRSDKTLKFTRMQKAGFLYYEDLVSRVTRAEAEAVSVLVKEAVWAFLPDAFVTMTGGFRLGKKIGHDVDFLITSPGSTEEEEQQLLHKVINLWEKKGLLLYYDLVESTFEKLKLPSRTVDALDHFQKCFLILKLHHQRVGSGKSSQQEGKTWKAIRVDLVMCPYERRAFALLGWTGSPQFNRDLRRYATHERKMMLDNHALYDKTKRIFLKAESEEEIFAHLGLDYIEPWERNA

SEQ ID NO: 48 - protein, 362 aa, artificial sequence
  N35 trunc new
KISEYACQRRTTLNNYNEIFTRAFEVLAENYEFRENEESYVTFRRAASVLKSLPFTIISMKDTEGIPCLGDKVKRVIEEIIEDGESSEVKAVLNDERYQAFKLFTSVFGVGRKTSEKWFRMGFRTLEKIRSDKTLKFTRMQKAGFLYYEDLAERVTRAEAEAVSVLVKEAVWAFLPDAFVTMTGGFRLGKKIGHDVDFLITSPGSTEEEEQQLLPKVINLWERKGLLLYYDLVESTFEKLKLPSRKVDALDHFQKCFLILKLHHQRVGSGKSSQQEGKTWKAIRVDLVMCPYERRAFALLGWTGSAFFNRDLRRYATHERKMILDNHALYDKTKRIFLKAESEEEIFAHLGLDYIEPWERNA

SEQ ID NO: 49 - protein, 361 aa, Bubalus bubalis
KISQYACQRKTTLNNYNHIFTDAFEILAENSEFKENEVSYVTFMRAASVLKSLPFTIISMKDTQGIPCLGDKVKCVIEEIIEDGESSEVKAVLNDERYQSFKLFTSVFGVGLKTSEKWFRMGFRSLSKITSDKTLKFTKMQKAGFLYYEDLVSCVTRAEAEAVGVLVKEAVWAFLPDAFITMTGGFRRGKKIGHDVDFLITSPGSAEDEEQLLPKVINLWEKKGLLLYYDLVESTFEKFKLPSRQVDTLDHFQKCFLILKLHHQRVDSGRSNQQEGKTWKAIRVDLVMCPYENRAFALLGWTGSRQFERDIRRYATHERKMMLDNHALYDKTKRVFLKAESEEEIFAHLGLDYIEPWERNA

SEQ ID NO: 50 - protein, 362 aa, Marmota flaviventris
TISQYACQRRTTLNNCNRVFTDAFDVLAENYEFRENESCSVVFMRAASVLKSLPFTIISMRDLEGIPCLEGKAKSIIEEIIEDGESSEVKAVLNDERYKSFKLFTSVFGVGLKTSEKWFRMGFRTLSKIRSDKSLKFTHMQKAGFLYYEDLVSCVTRAEAEAVSVLVKEAVWAFLPDAFITMTGGFRRGKNIGHDVDFLITSAEATEEEEQQLLHKVTNLWEKKGLLLYCDLVESTFEKLKTPSRKVDALDHFQKCFLILKLHHQRVDSDKASQQGGKNWKAIRVDLVMCPYERRAFALLGWTGSRQFERDLRRYATHERKMILDNHALYDKTKRIFLKAESEEEIFAHLGLDYIEPWERNA

SEQ ID NO: 51 - protein, 362 aa, mouse
KISEYACQRRTTLNNYNELFTRALDILAENDEFRENEESRDAFRRASSVLKSLPFPITSMKDTEGIPCLGDKVKRIIEEIIEDGESSEVKAVLNDERYKAFKLFTSVFGVGRKTAEKWFRMGFRTLEKIRSDKSLRFTQMQKAGFLYYEDLAERVNRPEAEAIRMLVKEAVVTFLPDALVTMTGGFRLGKMTGHDVDFLITSPEATEDEEQQLLHKVTDFWKQQGLLLYCDILESTFEKFKQPSRTVDALDHFQKCFLILKLDHPRVHSVKSGQQEGKGWKAIRVDLVMCPYDRRAFALLGWTGSPQFNRDLRRYATHERKMMLDNHALYDKTKRVFLEAESEEEIFAHLGLDYIEPWERNA

SEQ ID NO: 52 - protein, 361 aa, artificial sequence
  (M57 without His tag & linker) bovine-mouse chimera
KISEYACQRRTTLNNYNELFTRALDILAENDEFRENEESRDAFRRASSVLKSLPFPITSMKDTEGIPCLGDKVKRIIEEIIEDGESSEVKAVLNDERYKAFKLFTSVFGVGRKTAEKWFRMGFRTLEKIRSDKSLRFTQMQKAGFLYYEDLVSGVTRAEAEAVGVLVKEAVWAFLPDAFVTMTGGFRLGKKIGHDVDFLITSPGSAEDEEQLLPKVINLWEKKGLLLYYDLVESTFEKFKLPSRQVDTLDHFQKCFLILKLHHQRVDSSKSNQQEGKTWKAIRVDLVMCPYENRAFALLGWTGSPQFNRDLRRYATHERKMMLDNHALYDKTKRVFLEAESEEEIFAHLGLDYIEPWERNA

SEQ ID NO: 53 - protein, 361 aa, artificial sequence
  (M59 without His Tag and linker) bovine-mouse chimera
KISEYACQRRTTLNNYNELFTRALDILAENDEFRENEESRDAFRRASSVLKSLPFPITSMKDTEGIPCLGDKVKRIIEEIIEDGESSEVKAVLNDERYKAFKLFTSVFGVGRKTAEKWFRMGFRTLEKIRSDKSLRFTQMQKAGFLYYEDLAERVNRPEAEAIRMLVKEAVVTFLPDALVTMTGGFRLGKMTGHDVDFLITSPGSAEDEEQLLPKVINLWEKKGLLLYYDLVESTFEKFKLPSRQVDTLDHFQKCFLILKLHHQRVDSSKSNQQEGKTWKAIRVDLVMCPYENRAFALLGWTGSPQFNRDLRRYATHERKMMLDNHALYDKTKRVFLEAESEEEIFAHLGLDYIEPWERNA

SEQ ID NO: 54 - protein, 362 aa, mouse
KISEYACQRRTTLNNYNQLFTDALDILAENDEFRENEESCLAFRRASSVLKSLPFPITSMKDTEGIPCLGDKVKSIIEGIIEDGESSEVKAVLNDERYKSFKLFTSVFGVGLKTAEKWFRMGFRTLSKIQSDKSLRFTQMQKAGFLYYEDLVSGVNRPEAEAVSMLVKEAVVTFLPDALVTMTGGFRLGKMTGHDVDFLITSPEATEDEEQQLLHKVTDFWKQQGLLLYCDILESTFEKFKQPSRTVDALDHFQKCFLILKLDHPRVHSVKSGQQEGKGWKAIRVDLVMCPYDRRAFALLGWTGSPQFNRDLRRYATHERKMMLDNHALYDKTKRVFLEAESEEEIFAHLGLDYIEPWERNA

SEQ ID NO: 55 - protein, 361 aa, artificial sequence
  M54 (from 822)
KISEYACQRKTTLNNYNEIFTRAFEILAENSEFKENEESYVTFRRAASVLKSLPFTIISMKDTEGIPCLGDKVKRIIEEIIEDGESSEVKAVLNDERYQAFKLFTSVFGVGRKTSEKWFRMGFRSLEKIRSDKTLKFTKMQKAGFLYYEDLVSGVTRAEAEAVGVLVKEAVWAFLPDAFVTMTGGFRLGKKIGHDVDFLITSPGSAEDEEQLLPKVINLWEKKGLLLYYDLVESTFEKFKLPSRQVDTLDHFQKCFLILKLHHQRVDSSKSNQQEGKTWKAIRVDLVMCPYENRAFALLGWTGSAFFNRDIRRYATHERKMMLDNHALYDKTKRVFLKAESEEEIFAHLGLDYIEPRERNA

SEQ ID NO: 56 - protein, 362 aa, Artificial Sequence
  M77 without His tag
KKISEYACQRRTTLNNYNELFTRALDILAENDEFRENEESRDAFRRASSVLKSLPFPITSMKDTEGIPCLGDKVKRIIEEIIEDGESSEVKAVLNDERYKAFKLFTSVFGVGRKTAEKWFRMGFRTLEKIRSDKSLRFTQMQKAGFLYYEDLVSGVTRAEAEAVGVLVKEAVWAFLPDAFVTMTGGFRLGKKIGHDVDFLITSPGSAEDEEQLLPKVINLWEKKGLLLYYDLVESTFEKFKLPSRQVDTLDHFQKCFLILKLHHQRVDSSKSNQQEGKTWKAIRVDLVMCPYENRAFALLGWTGSPQFNRDLRRYATHERKMMLDNHALYDKTKRVFLEAESEEEIFAHLGLDYIEPWERNA

SEQ ID NO: 57 - protein, 377 aa, Artificial Sequence
  M77 with His tag
MASSHHHHHHSSGSEKKISEYACQRRTTLNNYNELFTRALDILAENDEFRENEESRDAFRRASSVLKSLPFPITSMKDTEGIPCLGDKVKRIIEEIIEDGESSEVKAVLNDERYKAFKLFTSVFGVGRKTAEKWFRMGFRTLEKIRSDKSLRFTQMQKAGFLYYEDLVSGVTRAEAEAVGVLVKEAVWAFLPDAFVTMTGGFRLGKKIGHDVDFLITSPGSAEDEEQLLPKVINLWEKKGLLLYYDLVESTFEKFKLPSRQVDTLDHFQKCFLILKLHHQRVDSSKSNQQEGKTWKAIRVDLVMCPYENRAFALLGWTGSPQFNRDLRRYATHERKMMLDNHALYDKTKRVFLEAESEEEIFAHLGLDYIEPWERNA

SEQ ID NO: 58 - protein, 361 aa, artificial sequence; identical to SEQ ID NO: 52
  C1-40 without His tag

SEQ ID NO: 59 - protein, 376 aa, artificial sequence
  C1-40 with His tag
MASSHHHHHHSSGSEKISEYACQRRTTLNNYNELFTRALDILAENDEFRENEESRDAFRRASSVLKSLPFPITSMKDTEGIPCLGDKVKRIIEEIIEDGESSEVKAVLNDERYKAFKLFTSVFGVGRKTAEKWFRMGFRTLEKIRSDKSLRFTQMQKAGFLYYEDLVSGVTRAEAEAVGVLVKEAVWAFLPDAFVTMTGGFRLGKKIGHDVDFLITSPGSAEDEEQLLPKVINLWEKKGLLLYYDLVESTFEKFKLPSRQVDTLDHFQKCFLILKLHHQRVDSSKSNQQEGKTWKAIRVDLVMCPYENRAFALLGWTGSPQFNRDLRRYATHERKMMLDNHALYDKTKRVFLEAESEEEIFAHLGLDYIEPWERNA

SEQ ID NO: 60 - protein, 363 aa, artificial sequence
  A2-20 without His tag
VTTVSEYACQRRTTLNNYNELFTRALDILAENDEFRENEESRDAFRRASSVLKSLPFPITSMKDTEGIPCLGDKVKRIIEEIIEDGESSEVKAVLNDERYKAFKLFTSVFGVGRKTAEKWFRMGFRTLEKIRSDKSLRFTQMQKAGFLYYEDLVSGVTRAEAEAVGVLVKEAVWAFLPDAFVTMTGGFRLGKKIGHDVDFLITSPGSAEDEEQLLPKVINLWEKKGLLLYYDLVESTFEKFKLPSRQVDTLDHFQKCFLILKLHHQRVDSSKSNQQEGKTWKAIRVDLVMCPYENRAFALLGWTGSPQFNRDLRRYATHERKMMLDNHALYDKTKRVFLEAESEEEIFAHLGLDYIEPWERNA

SEQ ID NO: 61 - protein, 379 aa, artificial sequence
  A2-20 with His tag
MASSHHHHHHSSGSENVTTVSEYACQRRTTLNNYNELFTRALDILAENDEFRENEESRDAFRRASSVLKSLPFPITSMKDTEGIPCLGDKVKRIIEEIIEDGESSEVKAVLNDERYKAFKLFTSVFGVGRKTAEKWFRMGFRTLEKIRSDKSLRFTQMQKAGFLYYEDLVSGVTRAEAEAVGVLVKEAVWAFLPDAFVTMTGGFRLGKKIGHDVDFLITSPGSAEDEEQLLPKVINLWEKKGLLLYYDLVESTFEKFKLPSRQVDTLDHFQKCFLILKLHHQRVDSSKSNQQEGKTWKAIRVDLVMCPYENRAFALLGWTGSPQFNRDLRRYATHERKMMLDNHALYDKTKRVFLEAESEEEIFAHLGLDYIEPWERNA

SEQ ID NO: 62 - protein, 363 aa, artificial sequence
  ii-ell-40 without His tag
VATVSEYACQRRTTLNNYNELFTRALDILAENDEFRENEESRDAFRRASSVLKSLPFPITSMKDTEGIPCLGDKVKRIIEEIIEDGESSEVKAVLNDERYKAFKLFTSVFGVGRKTAEKWFRMGFRTLEKIRSDKSLRFTQMQKAGFLYYEDLVSGVTRAEAEAVGVLVKEAVWAFLPDAFVTMTGGFRLGKKIGHDVDFLITSPGSAEDEEQLLPKVINLWEKKGLLLYYDLVESTFEKFKLPSRQVDTLDHFQKCFLILKLHHQRVDSSKSNQQEGKTWKAIRVDLVMCPYENRAFALLGWTGSPQFNRDLRRYATHERKMMLDNHALYDKTKRVFLEAESEEEIFAHLGLDYIEPWERNA

SEQ ID NO: 63 - protein, 379 aa, artificial sequence
  ii-ell-40 with His tag
MASSHHHHHHSSGSENVATVSEYACQRRTTLNNYNELFTRALDILAENDEFRENEESRDAFRRASSVLKSLPFPITSMKDTEGIPCLGDKVKRIIEEIIEDGESSEVKAVLNDERYKAFKLFTSVFGVGRKTAEKWFRMGFRTLEKIRSDKSLRFTQMQKAGFLYYEDLVSGVTRAEAEAVGVLVKEAVWAFLPDAFVTMTGGFRLGKKIGHDVDFLITSPGSAEDEEQLLPKVINLWEKKGLLLYYDLVESTFEKFKLPSRQVDTLDHFQKCFLILKLHHQRVDSSKSNQQEGKTWKAIRVDLVMCPYENRAFALLGWTGSPQFNRDLRRYATHERKMMLDNHALYDKTKRVFLEAESEEEIFAHLGLDYIEPWERNA

SEQ ID NO: 64 - protein, 363 aa, artificial sequence; identical to SEQ ID NO: 62
  9-40 without His tag

SEQ ID NO: 65 - protein, 379 aa, artificial sequence; identical to SEQ ID NO: 63
  9-40 with His tag

SEQ ID NO: 66 - protein, 365 aa, artificial sequence
  (45-751)(loop2 his tag)
MAEKKISEYACQRRTTLNNYNELFTRALDILAENDEFRENEESRDAFRRASSVLKSLPFPITSMKDTEGIPCLGDKVKRIIEEIIEDGESSEVKAVLNDERYKAFKLFTSVFGVGRKTAEKWFRMGFRTLEEIRSDKSLRFTQMQKAGFLYYEDLVSGVTRAEAEAVGVLVKEAVWAFLPDAFVTMTGGFRLGKKIGHDVDFLITSPGSAEDEEQLLPKVINLWEKKGLLLYYDLVESTLEKFKLPSRQVDTLDHFQKCFLILKLHRQRVDSSKHHHHHHKTWKAIRVDLVMCPYENRAFALLGWTGSPQFNRDLRRYATHERKMMLDNHALYDKTKRVFLEAESEEEIFAHLGLDYIEPWERNA

SEQ ID NO: 67 - protein, 369 aa, Artificial Sequence
  (46-737)(loop2 his tag)
MAHHGSEKKISEYACQRRTTLNNYNELFTRALDILAENDEFRENEESRDAFRRASSVLKSLPFPITSMKDTEGIPCLGDKVKRIIEEIIEDGESSEVKAVLNDERYKAFKLFTSVFGVGRKTAEKWFRMGFRTLEEIRSDKSLRFTQMQKAGFLYYEDLVSGVTRAEAEAVGVLVKEAVWAFLPDAFVTMTGGFRLGKKIGHDVDFLITSPGSAEDEEQLLPKVINLWEKKGLLLYYDLVESTLEKFKRPSRQVDTLDHFQKCFLILKLHRQRVDSSKHHHHHHETWKAIRVDLVMCPYENRAFALLGWTGSPQFNRDLRRYATHERKMMLDNHALYDKTKRVFLEAESEEEIFAHLGLDYIEPWERNA

SEQ ID NO: 68 - protein, 361 aa, Artificial Sequence
  TdT-M96 without N-terminal His tag
KISEYACQRRTTLNNYNELFTRALDILAENDEFRENEESRDAFRRASSVLKSLPFPITSMKDTEGIPCLGDKVKRIIEEIIEDGESSEVKAVLNDERYKAFKLFTSVFGVGRKTAEKWFRMGFRTLEEIRSDKSLRFTQMQKAGFLYYEDLVSGVTRAEAEAVGVLVKEAVWAFLPDAFVTMTGGFRLGKKIGHDVDFLITSPGSAEDEEQLLPKVINLWEKKGLLLYYNLVESTFEKFKLPSRQVDTLDHFQKCFLILKLHHQRVDSSKSNQQEGKTWKAIRVDLVMCPYENRAFALLGWTGSPQFNRDLRRYATHERKMMLDNHALYDKTKRVFLEAESEEEIFAHLGLDYIEPWERNA

SEQ ID NO: 69 - protein, 377 aa, Artificial Sequence
  TdT-M96 with N-terminal His tag
MASSHHHHHHSSGSEKKISEYACQRRTTLNNYNELFTRALDILAENDEFRENEESRDAFRRASSVLKSLPFPITSMKDTEGIPCLGDKVKRIIEEIIEDGESSEVKAVLNDERYKAFKLFTSVFGVGRKTAEKWFRMGFRTLEEIRSDKSLRFTQMQKAGFLYYEDLVSGVTRAEAEAVGVLVKEAVWAFLPDAFVTMTGGFRLGKKIGHDVDFLITSPGSAEDEEQLLPKVINLWEKKGLLLYYNLVESTFEKFKLPSRQVDTLDHFQKCFLILKLHHQRVDSSKSNQQEGKTWKAIRVDLVMCPYENRAFALLGWTGSPQFNRDLRRYATHERKMMLDNHALYDKTKRVFLEAESEEEIFAHLGLDYIEPWERNA

SEQ ID NO: 70 - protein, 361 aa, Artificial Sequence
  TdT-M103 without N-terminal His tag
KISEYACQRRTTLNNYNELFTRALDILVENDEFRENEESRDAFRRASSVLKSLPFPITSMKDTEGIPCLGDKVKRIIEEIIEDGESSEVKAVLNDERYKAFKLFTSVFGVGRKTAEKWFRMGFRTLEKIRSDKSLRFTQMQKAGFLYYEDLVSGVTRAEAEAVGVLVKEAVWAFLPDAFVTMTGGFRLGKKIGHDVDFLITSPGSAEDEEQLLPKVINLWEKKGLLLYYDLRESTFEKFKLPSRQVDTLDHFQKCFLILKLHHQRVDSSKSNQQEGKTWKAIRVDLVMCPYENRAFALLGWTGSPQFNRDLRRYATHERKMMLDNHALYDKTKRVFLEAESEEEIFAHLGLDYIEPWERNA

SEQ ID NO: 71 - protein, 377 aa, Artificial Sequence
  TdT-M103 with N-terminal His tag
MASSHHHHHHSSGSEKKISEYACQRRTTLNNYNELFTRALDILVENDEFRENEESRDAFRRASSVLKSLPFPITSMKDTEGIPCLGDKVKRIIEEIIEDGESSEVKAVLNDERYKAFKLFTSVFGVGRKTAEKWFRMGFRTLEKIRSDKSLRFTQMQKAGFLYYEDLVSGVTRAEAEAVGVLVKEAVWAFLPDAFVTMTGGFRLGKKIGHDVDFLITSPGSAEDEEQLLPKVINLWEKKGLLLYYDLRESTFEKFKLPSRQVDTLDHFQKCFLILKLHHQRVDSSKSNQQEGKTWKAIRVDLVMCPYENRAFALLGWTGSPQFNRDLRRYATHERKMMLDNHALYDKTKRVFLEAESEEEIFAHLGLDYIEPWERNA